European Patent Application EP 4 269 437 A1, published November 1, 2023. Title: PD-1 BINDING MOLECULE AND APPLICATION THEREOF. Applicant: ZHEJIANG NANOMAB TECH CENTER CO LTD. The sequence listing filed with the application follows.

SEQUENCE LISTING (327 sequences)

SEQ ID NO: 1 - protein, 8 aa, Artificial Sequence
  CDR1
  misc_feature (2)..(2): Xaa is Asp, Phe, Gly, His, Leu or Arg
  misc_feature (3)..(3): Xaa is Pro, Ser or Thr
  misc_feature (4)..(4): Xaa is Ala, Phe, Ile, Leu, Asn, Arg, Ser or Val
  misc_feature (5)..(5): Xaa is Asp, Phe, Gly, Leu, Met, Asn or Ser
  misc_feature (6)..(6): Xaa is Ala, Asp, Phe, Gly, Ile, Asn, Arg, Ser or Thr
  misc_feature (7)..(7): Xaa is Asp, Phe, His, Ile, Leu, Ser, Val, Trp or Tyr
  misc_feature (8)..(8): Xaa is Ala, Asp, Glu, Gly, Asn, Pro, Ser or Thr
GXXXXXXX

SEQ ID NO: 2 - protein, 9 aa, Artificial Sequence
  CDR2
  misc_feature (1)..(1): Xaa is Ile, Leu, Ser, Thr or Val
  misc_feature (2)..(2): Xaa is Ala, Asn, Ser or Thr
  misc_feature (3)..(3): Xaa is Phe, Gly, Ile, Lys, Leu, Met, Asn, Gln, Arg, Ser, Thr, Trp or Tyr
  misc_feature (4)..(4): Xaa is Ala, Asp, Gly, His, Asn, Arg, Ser or Thr
  misc_feature (5)..(5): Xaa is Ala, Asp, Gly, Asn, Arg, Ser or null
  misc_feature (6)..(6): Xaa is Gly, Arg, Ser or Thr
  misc_feature (7)..(7): Xaa is Asp, Glu, Ile, Leu, Met, Asn, Arg, Ser, Thr or Val
  misc_feature (8)..(8): Xaa is Ala, Lys, Met, Gln or Thr
  misc_feature (9)..(9): Xaa is Ala or null
XXXXXXXXX

SEQ ID NO: 3 - protein, 22 aa, Artificial Sequence
  CDR3
  misc_feature (1)..(1): Xaa is Ala, Glu, Gly, Asn, Arg, Ser, Thr or Val
  misc_feature (2)..(2): Xaa is Ala, Gly, Ile, Lys, Leu, Pro, Arg, Thr or Val
  misc_feature (3)..(3): Xaa is Ala, Asp, Glu, Gly, Lys, Asn, Pro, Arg, Ser, Val or Tyr
  misc_feature (4)..(4): Xaa is Ala, Cys, Asp, Glu, Gly, Ile, Lys, Leu, Arg, Ser, Thr, Val or Tyr
  misc_feature (5)..(5): Xaa is Ala, Cys, Asp, Phe, Gly, His, Ile, Lys, Leu, Asn, Pro, Gln, Arg, Ser, Trp or Tyr
  misc_feature (6)..(6): Xaa is Ala, Cys, Asp, Glu, Gly, Ile, Lys, Leu, Met, Pro, Gln, Arg, Ser or Tyr
  misc_feature (7)..(7): Xaa is Ala, Cys, Asp, Phe, Gly, His, Ile, Asn, Pro, Arg, Ser, Thr, Val or Tyr
  misc_feature (8)..(8): Xaa is Ala, Cys, Asp, Glu, Gly, Ile, Arg, Ser, Thr, Val, Trp, Tyr or null
  misc_feature (9)..(9): Xaa is Ala, Asp, Glu, Phe, Gly, Ile, Leu, Pro, Arg, Ser, Val, Trp, Tyr or null
  misc_feature (10)..(10): Xaa is Cys, Asp, Phe, Gly, Lys, Leu, Asn, Pro, Arg, Ser, Thr, Val, Trp, Tyr or null
  misc_feature (11)..(11): Xaa is Asp, Phe, Gly, His, Ile, Lys, Leu, Asn, Pro, Ser, Thr, Val, Tyr or null
  misc_feature (12)..(12): Xaa is Ala, Asp, Gly, His, Ile, Leu, Met, Pro, Arg, Ser, Thr, Val, Tyr or null
  misc_feature (13)..(13): Xaa is Cys, Asp, Glu, His, Pro, Arg, Ser, Thr, Val, Tyr or null
  misc_feature (14)..(14): Xaa is Ala, Asp, Glu, Phe, His, Ile, Leu, Pro, Arg, Thr, Tyr or null
  misc_feature (15)..(15): Xaa is Ala, Asp, Glu, Gly, Asn, Gln, Arg, Ser, Thr, Val, Tyr or null
  misc_feature (16)..(16): Xaa is Ala, Asp, Glu, Phe, Gly, His, Met, Pro, Ser, Val, Tyr or null
  misc_feature (17)..(17): Xaa is Ala, Asp, Glu, His, Asn, Gln, Arg, Thr, Tyr or null
  misc_feature (18)..(18): Xaa is Asp, Glu, Arg, Ser, Tyr or null
  misc_feature (19)..(19): Xaa is Asn, Ser, Tyr or null
  misc_feature (20)..(20): Xaa can be any naturally occurring amino acid
  misc_feature (21)..(21): Xaa is Glu, Asn, Tyr or null
  misc_feature (22)..(22): Xaa is Tyr or null
XXXXXXXXXXXXXXXXXXXXXX

SEQ ID NO: 4 - protein, 8 aa, Artificial Sequence
  CDR1
GDTALISA

SEQ ID NO: 5 - protein, 8 aa, Artificial Sequence
  CDR1
GRTFSSVA

SEQ ID NO: 6 - protein, 8 aa, Artificial Sequence
  CDR1
GGTFSGSE

SEQ ID NO: 7 - protein, 8 aa, Artificial Sequence
  CDR1
GRTFSSYG

SEQ ID NO: 8 - protein, 8 aa, Artificial Sequence
  CDR1
GGTFSGYG

SEQ ID NO: 9 - protein, 8 aa, Artificial Sequence
  CDR1
GRTFMRYS

SEQ ID NO: 10 - protein, 8 aa, Artificial Sequence
  CDR1
GRTFSSYA

SEQ ID NO: 11 - protein, 8 aa, Artificial Sequence
  CDR1
GDTILISS

SEQ ID NO: 12 - protein, 8 aa, Artificial Sequence
  CDR1
GFTFSSYP

SEQ ID NO: 13 - protein, 8 aa, Artificial Sequence
  CDR1
GGTFGRLE

SEQ ID NO: 14 - protein, 8 aa, Artificial Sequence
  CDR1
GDTRLASA

SEQ ID NO: 15 - protein, 8 aa, Artificial Sequence
  CDR1
GRSFNSYA

SEQ ID NO: 16 - protein, 8 aa, Artificial Sequence
  CDR1
GDTSFISA

SEQ ID NO: 17 - protein, 8 aa, Artificial Sequence
  CDR1
GGTFNSYA

SEQ ID NO: 18 - protein, 8 aa, Artificial Sequence
  CDR1
GRTFNGYG

SEQ ID NO: 19 - protein, 8 aa, Artificial Sequence
  CDR1
GRPFSIYD

SEQ ID NO: 20 - protein, 8 aa, Artificial Sequence
  CDR1
GDTILISA

SEQ ID NO: 21 - protein, 8 aa, Artificial Sequence
  CDR1
GDTNLFSA

SEQ ID NO: 22 - protein, 8 aa, Artificial Sequence
  CDR1
GFTLDDHS

SEQ ID NO: 23 - protein, 8 aa, Artificial Sequence
  CDR1
GRTFNSYA

SEQ ID NO: 24 - protein, 8 aa, Artificial Sequence
  CDR1
GRTFSSVP

SEQ ID NO: 25 - protein, 8 aa, Artificial Sequence
  CDR1
GDTALFSA

SEQ ID NO: 26 - protein, 8 aa, Artificial Sequence
  CDR1
GRTFSGYT

SEQ ID NO: 27 - protein, 8 aa, Artificial Sequence
  CDR1
GGTISGYE

SEQ ID NO: 28 - protein, 8 aa, Artificial Sequence
  CDR1
GRTFSSIA

SEQ ID NO: 29 - protein, 8 aa, Artificial Sequence
  CDR1
GGTFSNFN

SEQ ID NO: 30 - protein, 8 aa, Artificial Sequence
  CDR1
GRTFSSYN

SEQ ID NO: 31 - protein, 8 aa, Artificial Sequence
  CDR1
GFSVGDYS

SEQ ID NO: 32 - protein, 8 aa, Artificial Sequence
  CDR1
GFTFSSWA

SEQ ID NO: 33 - protein, 8 aa, Artificial Sequence
  CDR1
GDTILFSA

SEQ ID NO: 34 - protein, 8 aa, Artificial Sequence
  CDR1
GFTLDDYS

SEQ ID NO: 35 - protein, 8 aa, Artificial Sequence
  CDR1
GFTFSSDA

SEQ ID NO: 36 - protein, 8 aa, Artificial Sequence
  CDR1
GRTFSGYA

SEQ ID NO: 37 - protein, 8 aa, Artificial Sequence
  CDR1
GHSFSIYD

SEQ ID NO: 38 - protein, 8 aa, Artificial Sequence
  CDR1
GGPFSIYD

SEQ ID NO: 39 - protein, 8 aa, Artificial Sequence
  CDR1
GLTFSTYA

SEQ ID NO: 40 - protein, 7 aa, Artificial Sequence
  CDR2
LTNTGIT

SEQ ID NO: 41 - protein, 8 aa, Artificial Sequence
  CDR2
ISRSGGSA

SEQ ID NO: 42 - protein, 8 aa, Artificial Sequence
  CDR2
ISRNGGTT

SEQ ID NO: 43 - protein, 7 aa, Artificial Sequence
  CDR2
ITNTGLT

SEQ ID NO: 44 - protein, 8 aa, Artificial Sequence
  CDR2
ISRHGGST

SEQ ID NO: 45 - protein, 8 aa, Artificial Sequence
  CDR2
ISWGGSST

SEQ ID NO: 46 - protein, 8 aa, Artificial Sequence
  CDR2
INGNGRSQ

SEQ ID NO: 47 - protein, 7 aa, Artificial Sequence
  CDR2
ITNSGLT

SEQ ID NO: 48 - protein, 8 aa, Artificial Sequence
  CDR2
LTGAGGST

SEQ ID NO: 49 - protein, 7 aa, Artificial Sequence
  CDR2
ISWDGET

SEQ ID NO: 50 - protein, 8 aa, Artificial Sequence
  CDR2
VSMSGRTT

SEQ ID NO: 51 - protein, 8 aa, Artificial Sequence
  CDR2
ISQNGGTQ

SEQ ID NO: 52 - protein, 7 aa, Artificial Sequence
  CDR2
ITNTGIT

SEQ ID NO: 53 - protein, 8 aa, Artificial Sequence
  CDR2
INLSRGNT

SEQ ID NO: 54 - protein, 8 aa, Artificial Sequence
  CDR2
ISWRDSSK

SEQ ID NO: 55 - protein, 8 aa, Artificial Sequence
  CDR2
INLSRGDT

SEQ ID NO: 56 - protein, 7 aa, Artificial Sequence
  CDR2
ITNSGVT

SEQ ID NO: 57 - protein, 7 aa, Artificial Sequence
  CDR2
ITNSGMT

SEQ ID NO: 58 - protein, 8 aa, Artificial Sequence
  CDR2
ISTSDGRT

SEQ ID NO: 59 - protein, 8 aa, Artificial Sequence
  CDR2
ISQNGGSQ

SEQ ID NO: 60 - protein, 8 aa, Artificial Sequence
  CDR2
ISKSGGSA

SEQ ID NO: 61 - protein, 8 aa, Artificial Sequence
  CDR2
ISYSGGST

SEQ ID NO: 62 - protein, 8 aa, Artificial Sequence
  CDR2
ISRNGRST

SEQ ID NO: 63 - protein, 8 aa, Artificial Sequence
  CDR2
INWSGRSQ

SEQ ID NO: 64 - protein, 8 aa, Artificial Sequence
  CDR2
SNWSAGTT

SEQ ID NO: 65 - protein, 8 aa, Artificial Sequence
  CDR2
VNWSNSSA

SEQ ID NO: 66 - protein, 8 aa, Artificial Sequence
  CDR2
ISWSGGSQ

SEQ ID NO: 67 - protein, 8 aa, Artificial Sequence
  CDR2
TARDSGST

SEQ ID NO: 68 - protein, 9 aa, Artificial Sequence
  CDR2
ISSGSGEMA

SEQ ID NO: 69 - protein, 8 aa, Artificial Sequence
  CDR2
TSNRDGST

SEQ ID NO: 70 - protein, 8 aa, Artificial Sequence
  CDR2
ITIDGGST

SEQ ID NO: 71 - protein, 8 aa, Artificial Sequence
  CDR2
VNWRNTTA

SEQ ID NO: 72 - protein, 8 aa, Artificial Sequence
  CDR2
ISLSRGNT

SEQ ID NO: 73 - protein, 8 aa, Artificial Sequence
  CDR2
INLARGNT

SEQ ID NO: 74 - protein, 8 aa, Artificial Sequence
  CDR2
VTLSRGNT

SEQ ID NO: 75 - protein, 8 aa, Artificial Sequence
  CDR3
INFGRGTT

SEQ ID NO: 76 - protein, 17 aa, Artificial Sequence
  CDR3
NAGAPPPGGLGYDESDY

SEQ ID NO: 77 - protein, 16 aa, Artificial Sequence
  CDR3
AASELDFCSTLGCYDY

SEQ ID NO: 78 - protein, 22 aa, Artificial Sequence
  CDR3
AAGLRAYYGDSYVDTMTENYNY

SEQ ID NO: 79 - protein, 22 aa, Artificial Sequence
  CDR3
AAALRPDYGDSYVYTSTSNYEY

SEQ ID NO: 80 - protein, 21 aa, Artificial Sequence
  CDR3
AADTNPSGSWDRPTNEAEYDY

SEQ ID NO: 81 - protein, 18 aa, Artificial Sequence
  CDR3
AAEGHLGVPTVRSDEYDY

SEQ ID NO: 82 - protein, 17 aa, Artificial Sequence
  CDR3
NAGGPPPGGLGYDESDY

SEQ ID NO: 83 - protein, 13 aa, Artificial Sequence
  CDR3
NAPAAMRDYGIDY

SEQ ID NO: 84 - protein, 11 aa, Artificial Sequence
  CDR3
AARVILRAYKY

SEQ ID NO: 85 - protein, 19 aa, Artificial Sequence
  CDR3
AAGRAQAEIPIMRAQEYDS

SEQ ID NO: 86 - protein, 21 aa, Artificial Sequence
  CDR3
AADGDASDISYAPPRDYEYDY

SEQ ID NO: 87 - protein, 17 aa, Artificial Sequence
  CDR3
GVDRRQYGLGIPPLADH

SEQ ID NO: 88 - protein, 16 aa, Artificial Sequence
  CDR3
RPYSDYVTYDPYDYDA

SEQ ID NO: 89 - protein, 17 aa, Artificial Sequence
  CDR3
NAGAPPPGGFGYDESDY

SEQ ID NO: 90 - protein, 16 aa, Artificial Sequence
  CDR3
TTDVACYSDYDPSFRF

SEQ ID NO: 91 - protein, 21 aa, Artificial Sequence
  CDR3
AADGDASDRSYAPPRDYEYEY

SEQ ID NO: 92 - protein, 16 aa, Artificial Sequence
  CDR3
AASSFDFCSTHGCYDY

SEQ ID NO: 93 - protein, 18 aa, Artificial Sequence
  CDR3
NRVIRGTRDPSIYYVMDY

SEQ ID NO: 94 - protein, 22 aa, Artificial Sequence
  CDR3
AAGLKADYGDSYVDTSTRNYNY

SEQ ID NO: 95 - protein, 16 aa, Artificial Sequence
  CDR3
AASSYDFCSTHGCYDY

SEQ ID NO: 96 - protein, 16 aa, Artificial Sequence
  CDR3
AASDYDFCSTHGCYDY

SEQ ID NO: 97 - protein, 18 aa, Artificial Sequence
  CDR3
AAERHLGVPTVRDDEYDD

SEQ ID NO: 98 - protein, 16 aa, Artificial Sequence
  CDR3
AASEYDFCSTHGCYDY

SEQ ID NO: 99 - protein, 18 aa, Artificial Sequence
  CDR3
NRVIRGTTYPDVYYGMDY

SEQ ID NO: 100 - protein, 16 aa, Artificial Sequence
  CDR3
RPYSDYVTYDPDDYDY

SEQ ID NO: 101 - protein, 21 aa, Artificial Sequence
  CDR3
AAKYHSGSYYYTSIRPEEYDY

SEQ ID NO: 102 - protein, 7 aa, Artificial Sequence
  CDR3
RVNSQDY

SEQ ID NO: 103 - protein, 10 aa, Artificial Sequence
  CDR3
AKGGYLTYAN

SEQ ID NO: 104 - protein, 17 aa, Artificial Sequence
  CDR3
NAGAPPPGEFGYDESDY

SEQ ID NO: 105 - protein, 15 aa, Artificial Sequence
  CDR3
STDCSLYGSTYSPDY

SEQ ID NO: 106 - protein, 13 aa, Artificial Sequence
  CDR3
NADRGIIIYGKTY

SEQ ID NO: 107 - protein, 16 aa, Artificial Sequence
  CDR3
RPYSDYVSYDPTEYDS

SEQ ID NO: 108 - protein, 17 aa, Artificial Sequence
  CDR3
GVDRRQYGWGIPPLADH

SEQ ID NO: 109 - protein, 17 aa, Artificial Sequence
  CDR3
GVDRRQYGLCIPPLADH

SEQ ID NO: 110 - protein, 17 aa, Artificial Sequence
  CDR3
GVDRRQYGLDIPPLADH

SEQ ID NO: 111 - protein, 17 aa, Artificial Sequence
  CDR3
GVDRRQYGLGIPHLADH

SEQ ID NO: 112 - protein, 17 aa, Artificial Sequence
  CDR3
GLDRIQYGLGIPPLADH

SEQ ID NO: 113 - protein, 17 aa, Artificial Sequence
  CDR3
GVDRRQYGLGSPPLADH

SEQ ID NO: 114 - protein, 17 aa, Artificial Sequence
  CDR3
GVDRRQDGLGIPPLADH

SEQ ID NO: 115 - protein, 17 aa, Artificial Sequence
  CDR3
GVGRRQYGLGIPPLADH

SEQ ID NO: 116 - protein, 17 aa, Artificial Sequence
  CDR3
GVDRRKYGLGIPPLADH

SEQ ID NO: 117 - protein, 17 aa, Artificial Sequence
  CDR3
GVDRRQYGLGIPPPADH

SEQ ID NO: 118 - protein, 17 aa, Artificial Sequence
  CDR3
GVERRQYGLGIPPLADH

SEQ ID NO: 119 - protein, 17 aa, Artificial Sequence
  CDR3
GVDRRQYGFGIPPLADH

SEQ ID NO: 120 - protein, 17 aa, Artificial Sequence
  CDR3
GVDRRQYGLGLPPLADH

SEQ ID NO: 121 - protein, 17 aa, Artificial Sequence
  CDR3
GVDRRQYGLGIPPLADY

SEQ ID NO: 122 - protein, 17 aa, Artificial Sequence
  CDR3
GVDSRQYGLGIPPLADH

SEQ ID NO: 123 - protein, 17 aa, Artificial Sequence
  CDR3
GVDRRQYGLGTPPLADH

SEQ ID NO: 124 - protein, 17 aa, Artificial Sequence
  CDR3
GVDRRQYGLGITPLADH

SEQ ID NO: 125 - protein, 17 aa, Artificial Sequence
  CDR3
GVDRRQYRLGIPPLADH

SEQ ID NO: 126 - protein, 17 aa, Artificial Sequence
  CDR3
GVDRRQYGLGNPPLADH

SEQ ID NO: 127 - protein, 17 aa, Artificial Sequence
  CDR3
GVDRRQYGLGIPPLAEH

SEQ ID NO: 128 - protein, 17 aa, Artificial Sequence
  CDR3
GVDRRQYGLGILPLADH

SEQ ID NO: 129 - protein, 17 aa, Artificial Sequence
  CDR3
GVDRRQYGLGIHPLADH

SEQ ID NO: 130 - protein, 17 aa, Artificial Sequence
  CDR3
GVDRRQYGLGVPPLADH

SEQ ID NO: 131 - protein, 17 aa, Artificial Sequence
  CDR3
GVVRRQYGLGIPPLADH

SEQ ID NO: 132 - protein, 17 aa, Artificial Sequence
  CDR3
GVDRRQYGLGISPLADH

SEQ ID NO: 133 - protein, 17 aa, Artificial Sequence
  CDR3
EVDRRQYGLGIPPLADH

SEQ ID NO: 134 - protein, 17 aa, Artificial Sequence
  CDR3
GVDKRQYGLGIPPLADH

SEQ ID NO: 135 - protein, 17 aa, Artificial Sequence
  CDR3
GIDRRQYGLGIPPLADH

SEQ ID NO: 136 - protein, 17 aa, Artificial Sequence
  CDR3
GVDRRRYGLGIPPLADH

SEQ ID NO: 137 - protein, 17 aa, Artificial Sequence
  CDR3
GVDRRQYGSGIPPLADH

SEQ ID NO: 138 - protein, 17 aa, Artificial Sequence
  CDR3
GVDGRQYGLGIPPLADH

SEQ ID NO: 139 - protein, 17 aa, Artificial Sequence
  CDR3
GVDRRQHGLGIPPLADH

SEQ ID NO: 140 - protein, 17 aa, Artificial Sequence
  CDR3
GVDRRQYWLGIPPLADH

SEQ ID NO: 141 - protein, 17 aa, Artificial Sequence
  CDR3
GVDRQQYGLGIPPLADH

SEQ ID NO: 142 - protein, 17 aa, Artificial Sequence
  CDR3
GVDRWQYGLGIPPLADH

SEQ ID NO: 143 - protein, 17 aa, Artificial Sequence
  CDR3
GGDRRQYGLGIPPLADH

SEQ ID NO: 144 - protein, 17 aa, Artificial Sequence
  CDR3
GVNRRQYGLGIPPLADH

SEQ ID NO: 145 - protein, 17 aa, Artificial Sequence
  CDR3
VVDRRQYGLGIPPLADH

SEQ ID NO: 146 - protein, 17 aa, Artificial Sequence
  CDR3
GVDRRQYGLRIPPLADH

SEQ ID NO: 147 - protein, 17 aa, Artificial Sequence
  CDR3
GVDRRQYGLGIPPLAAH

SEQ ID NO: 148 - protein, 17 aa, Artificial Sequence
  CDR3
GVDRRQYGLGIPTLADH

SEQ ID NO: 149 - protein, 17 aa, Artificial Sequence
  CDR3
GVDRLQYGLGIPPLADH

SEQ ID NO: 150 - protein, 17 aa, Artificial Sequence
  CDR3
GVDRRQYGLGIRPLADH

SEQ ID NO: 151 - protein, 17 aa, Artificial Sequence
  CDR3
GVDRRQYGLGFPPLADH

SEQ ID NO: 152 - protein, 17 aa, Artificial Sequence
  CDR3
GADRRQYGLGIPPLADH

SEQ ID NO: 153 - protein, 17 aa, Artificial Sequence
  CDR3
GVDRRQYGLSIPPLADH

SEQ ID NO: 154 - protein, 17 aa, Artificial Sequence
  CDR3
GVDIRQYGLGIPPLADH

SEQ ID NO: 155 - protein, 17 aa, Artificial Sequence
  CDR3
GVDKIQYGLGLPVLADH

SEQ ID NO: 156 - protein, 17 aa, Artificial Sequence
  CDR3
GVDRRQYGLGIPPRADH

SEQ ID NO: 157 - protein, 17 aa, Artificial Sequence
  CDR3
GVDRRQYGLGIPPFADH

SEQ ID NO: 158 - protein, 17 aa, Artificial Sequence
  CDR3
GVDRRQYGLGIPPLADR

SEQ ID NO: 159 - protein, 17 aa, Artificial Sequence
  CDR3
GVDRRQYGLGIPPLAGH

SEQ ID NO: 160 - protein, 17 aa, Artificial Sequence
  CDR3
GVDRRQYGVGIPPLADH

SEQ ID NO: 161 - protein, 17 aa, Artificial Sequence
  CDR3
GVDRRQYGLGIPPHADH

SEQ ID NO: 162 - protein, 17 aa, Artificial Sequence
  CDR3
GVARRQYGLGIPPLADH

SEQ ID NO: 163 - protein, 17 aa, Artificial Sequence
  CDR3
GVYRRQYGLGIPPLADH

SEQ ID NO: 164 - protein, 17 aa, Artificial Sequence
  CDR3
GVDRCQYGLGIPPLADH

SEQ ID NO: 165 - protein, 17 aa, Artificial Sequence
  CDR3
GVDRRQCGLGIPPLADH

SEQ ID NO: 166 - protein, 17 aa, Artificial Sequence
  CDR3
GVDRRQYGLGIPPLVDH

SEQ ID NO: 167 - protein, 17 aa, Artificial Sequence
  CDR3
GVDRRPYGLGIPPLADH

SEQ ID NO: 168 - protein, 17 aa, Artificial Sequence
  CDR3
GVDRRQYGLGIPPLADN

SEQ ID NO: 169 - protein, 17 aa, Artificial Sequence
  CDR3
GLDRIQYGLGIPPLADY

SEQ ID NO: 170 - protein, 17 aa, Artificial Sequence
  CDR3
GLDRRQYGLGIPPLADH

SEQ ID NO: 171 - protein, 17 aa, Artificial Sequence
  CDR3
GVDRRQYGLGIPPLADQ

SEQ ID NO: 172 - protein, 17 aa, Artificial Sequence
  CDR3
GVDRRQYGLGIPPIADH

SEQ ID NO: 173 - protein, 17 aa, Artificial Sequence
  CDR3
GVDRRQYGLVIPPLADH

SEQ ID NO: 174 - protein, 17 aa, Artificial Sequence
  CDR3
GVDRRQYVLGIPPLADH

SEQ ID NO: 175 - protein, 17 aa, Artificial Sequence
  CDR3
GVDRRQYGLGIPPLSDH

SEQ ID NO: 176 - protein, 17 aa, Artificial Sequence
  CDR3
GIDRIQYGLGIPPLADH

SEQ ID NO: 177 - protein, 17 aa, Artificial Sequence
  CDR3
GVDRREYGLGIPPLADH

SEQ ID NO: 178 - protein, 17 aa, Artificial Sequence
  CDR3
GVDRRQYGLGIPSLADH

SEQ ID NO: 179 - protein, 17 aa, Artificial Sequence
  CDR3
GVDRRQYGLGIPPLAHH

SEQ ID NO: 180 - protein, 17 aa, Artificial Sequence
  CDR3
GVDRRQNGLGIPPLADH

SEQ ID NO: 181 - protein, 17 aa, Artificial Sequence
  CDR3
GVDRRQYGLGIPPLAVH

SEQ ID NO: 182 - protein, 17 aa, Artificial Sequence
  CDR3
GVDRRQYGWCIPPLADH

SEQ ID NO: 183 - protein, 17 aa, Artificial Sequence
  CDR3
GVDRRQYELGIPPLADH

SEQ ID NO: 184 - protein, 123 aa, Artificial Sequence
  VHH
EVQVVESGGGLVQTGGSLRLSCAASGDTALISAMGWYRQAPGKERELVAALTNTGITYYADSVKGRFTISRDNAKNTVYLQMNSLKPEDTAVYYCNAGAPPPGGLGYDESDYWGQGTQVTVSS

SEQ ID NO: 185 - protein, 123 aa, Artificial Sequence
  VHH
EVQVVESGGGVVQAGDSLRLSCVASGRTFSSVAMGWFRQAPGKEREFVAAISRSGGSAGYSDSVKDRSTISRDNAKNTVYLQMNSLKPEDTAVYFCAASELDFCSTLGCYDYWGQGIQVTFSS

SEQ ID NO: 186 - protein, 129 aa, Artificial Sequence
  VHH
QVQLVESGGGLVQAGGSLRLSCAASGGTFSGSELGWFRQAPGKEREFVAGISRNGGTTGYSDSVKDRFTIARDNAKNTVYLQMNSLKPEDTAVYYCAAGLRAYYGDSYVDTMTENYNYWGQGTQVTVSS

SEQ ID NO: 187 - protein, 123 aa, Artificial Sequence
  VHH
DVQLQESGGGLVQAGGSLRVSCAASGRTFSSYGMGWFRQAPGKERELVAAITNTGLTYYADSVEGRFTISRDAAKNTVYLQMNSLEPEDTAVYYCNAGAPPPGGLGYDESDYWGQGTLVTVSS

SEQ ID NO: 188 - protein, 129 aa, Artificial Sequence
  VHH
QVQLVESGGGLVQAGDSLRLSCAASGGTFSGYGMGWFRQAPGKEREFVAGISRHGGSTGYSSSVKDRFTISRDNAKNTVDLQMNSLKPEDTAVYHCAAALRPDYGDSYVYTSTSNYEYWGQGTQVTVSS

SEQ ID NO: 189 - protein, 128 aa, Artificial Sequence
  VHH
QVQLVESGGGSVQAGDSLRISCEASGRTFMRYSMGWFRQASGKEREFVAAISWGGSSTYYADSVKGRFIISRDNTKNTVFLQMNSLKPEDTAVYYCAADTNPSGSWDRPTNEAEYDYWGQGTQVTVSS

SEQ ID NO: 190 - protein, 125 aa, Artificial Sequence
  VHH
QVQLVESGGGLLQAGDSLRLSCIASGRTFSSYAMGWFRQAPGKEREFVAGINGNGRSQYYAEVVKDRFFISRDNAKNTVYLQMNSLKPEDTAVYYCAAEGHLGVPTVRSDEYDYWGQGTQVTVSS

SEQ ID NO: 191 - protein, 123 aa, Artificial Sequence
  VHH
EVQVQESGGGLVQAGGSLTLSCAASGDTILISSIGWYRQAPGKERELVAAITNSGLTYYPDSVKGRFTISRDNAKNTVYLQMNNLKPEDTAVYYCNAGGPPPGGLGYDESDYWGQGTQVTVSS

SEQ ID NO: 192 - protein, 120 aa, Artificial Sequence
  VHH
QVQLVESGGGLVPPGGSLRLSCAASGFTFSSYPMSWYRQAPGRKRDFVAMLTGAGGSTDYADSVKGRFTISRDNAKNTVYLQMNSLKPEDTAVYYCNAPAAMRDYGIDYWGKGTLVNVSS

SEQ ID NO: 193 - protein, 117 aa, Artificial Sequence
  VHH
EVQLVESGGGLVQAGDSLRLSCAASGGTFGRLETGWFRQAPGKEREFVAAISWDGETSYADSVKGRFTISRDNAKNTMALQMNRLTPEDTAVYFCAARVILRAYKYWGQGTQVTVSS

SEQ ID NO: 194 - protein, 126 aa, Artificial Sequence
  VHH
QVQLVESGGGLVQAGGSLRLSCAASGRTFSSYAMGWFRQALGKEREWIAGVSMSGRTTYYAAPVKDRFTISRDNAKNTVTLQMNSLKPEDTAVYYCAAGRAQAEIPIMRAQEYDSWGQGTQVTVSS

SEQ ID NO: 195 - protein, 123 aa, Artificial Sequence
  VHH
EVQLVESGGGLVQAGGSLRLSCTASGDTRLASAMGWYRQAPGKERELVAVITNSGLTHYADSVEGRFTISRDSAKNTVYLQMNSLKPEDTAVYYCNAGAPPPGGLGYDESDYWDQGTQVTVSS

SEQ ID NO: 196 - protein, 128 aa, Artificial Sequence
  VHH
QVQLQESGGGLVQAGGSLRLSCAASGRSFNSYAMGWFRQAPGKEREFVAAISQNGGTQGYAEAVKDRFTISRDNTNKVVALQMNSLKPEDTAAYYCAADGDASDISYAPPRDYEYDYWGQGTQVTVSS

SEQ ID NO: 197 - protein, 123 aa, Artificial Sequence
  VHH
QVQLVESGGGLVQAGGSLRLSCAASGDTSFISAAGWYRQAPGKERELVAAITNTGITYYPDSVKGRFTISRDNAKNTVYLQMNNLKPEDTAVYYCNAGAPPPGGLGYDESDYWGQGTQVTVSS

SEQ ID NO: 198 - protein, 124 aa, Artificial Sequence
  VHH
QVKLEESGGGLVQAGGSLRLSCTASGGTFNSYAMGWFRQAPGKERESVAAINLSRGNTYYADSVKGRFTISRDNAKNTVYLQMNSLKPEDTAVYHCGVDRRQYGLGIPPLADHWGQGTQVTVSS

SEQ ID NO: 199 - protein, 123 aa, Artificial Sequence
  VHH
EVQLVESGGGLVQAGGSLRLSCAASGRTFNGYGMGWFRQAPGKEREFVAAISWRDSSKYYADSVRDRFTASRDNAKNTVYLQMNSLKPEDTAVYYCRPYSDYVTYDPYDYDAWGQGTQVTVSS

SEQ ID NO: 200 - protein, 124 aa, Artificial Sequence
  VHH
QVQLVETGGGLVRAGGSLRLSCTASGRPFSIYDMGWFRQAPDKERESVAVINLSRGDTYYADSVKGRFTISLDSAKNTVYLQMNSLKPEDTAVYSCGVDRRQYGLGIPPLADHWGQGTQVTVSS

SEQ ID NO: 201 - protein, 123 aa, Artificial Sequence
  VHH
EVQVVESGGGLVQAGGSLRLSCAASGDTILISAIGWYRQAPGKVRELVAAITNSGVTYYTDSVKGRFTISRDNAKNTVYLQMDSLKPEDTAVYYCNAGGPPPGGLGYDESDYWGPGTHVTVSS

SEQ ID NO: 202 - protein, 123 aa, Artificial Sequence
  VHH
QVQLVETGGGLVQAGGSLRLSCTASGDTNLFSAMGWHRQAPGKERELVAAITNSGMTYYADVVKGRFTLSRDNAKNTVYLQMNSLKPEDTAVYYCNAGAPPPGGFGYDESDYWGQGTQVTVSS

SEQ ID NO: 203 - protein, 123 aa, Artificial Sequence
  VHH
QVQLQESGGGLVQPGGSLRLSCAASGFTLDDHSIGWFRQAPGKEREPVSCISTSDGRTYYEDSVKGRFTISRDKAKNTVYLQMDSLKPEDTAVYYCTTDVACYSDYDPSFRFWGQGTQVTVSS

SEQ ID NO: 204 - protein, 128 aa, Artificial Sequence
  VHH
QVQLVESGGGLVQAGGSLTLSCAASGRTFNSYAMGWFRQAPGKEREFVAAISQNGGSQGYAEAVKDRFTISRDNTNKVVALQMNSLKPEDTAAYYCAADGDASDRSYAPPRDYEYEYWGQGTQVTVSS

SEQ ID NO: 205 - protein, 123 aa, Artificial Sequence
  VHH
EVQVVESGGGLVQAGGSLRLSCTASGDTRLASAMGWYRQAPGKERELVAAITNSGLTYYADSVEGRFTISRDSAKNTVYLQMNSLKPEDTAVYYCNAGAPPPGGLGYDESDYWGQGTQVTVSS

SEQ ID NO: 206 - protein, 123 aa, Artificial Sequence
  VHH
EVQLVESGGGLVQVGDSLRLSCAASGRTFSSVPMGWFRQAPGNQREFVAAISKSGGSAGYADSVKDRSTISRDNAKNTIYLQMNSLKPEDTAVYYCAASSFDFCSTHGCYDYWGQGTQVTISS

SEQ ID NO: 207 - protein, 123 aa, Artificial Sequence
  VHH
EVQVVESGGGLVQTGGSLRLSCAASGDTALFSAVGWYRQAPGKERELVAALTNTGITYYADSVEGRFTIFRDNAKNTVYLQMNSLKPEDTAVYYCNAGAPPPGGLGYDESDYWGQGTQVTVSS

SEQ ID NO: 208 - protein, 125 aa, Artificial Sequence
  VHH
EVQVVETGGGLAQAGGSLRLSCAASGRTFSGYTVGWYRQSPGKEREFVAAISYSGGSTDYADSVKGRFTISRDNANNTVYLQMGSLKAEDTAVYYCNRVIRGTRDPSIYYVMDYWGKGTLVTVSS

SEQ ID NO: 209 - protein, 129 aa, Artificial Sequence
  VHH
EVQVVESGGGLVQAGDSLRLSCAASGGTISGYEMGWFRQAPGKEREFVAGISRNGRSTGYSDSAKDRFTISRDNAKNTVYLQMNSLKPEDTAVYYCAAGLKADYGDSYVDTSTRNYNYWGQGTQVTVSS

SEQ ID NO: 210 - protein, 123 aa, Artificial Sequence
  VHH
QVQLVESGGGLVRAGDSLTLSCAASGRTFSSVPMGWFRQAPGNQREFVAAISKSGGSAGYADSVKDRSTISRDNAKNTIYLQMNSLKPEDTAVYYCAASSYDFCSTHGCYDYWGQGTQVTISS

SEQ ID NO: 211 - protein, 123 aa, Artificial Sequence
  VHH
QLQLVESGGGLVQAGDSLRLSCAASGRTFSSIAMGWFRQAPGKEREFVAAISRSGGSAGYADSVKDRSTIVRDNTKNTVYLQMNSLKPEDTAVYFCAASDYDFCSTHGCYDYWGQGTQVTISS

SEQ ID NO: 212 - protein, 125 aa, Artificial Sequence
  VHH
QVQLQESGGGLLQAGDSLRLSCIVSGRTFSSYAIGWFRQAPGKEREFVAGINWSGRSQYYSESVKDRFTVSIDNAKNTVYLQMNSLKPEDTAVYYCAAERHLGVPTVRDDEYDDWGQGTQVTVSS

SEQ ID NO: 213 - protein, 123 aa, Artificial Sequence
  VHH
EVQLVESGGGLVQAGDSLRLSCAASGRTFSSVAMGWFRQAPGKEREFVAAISRSGGSAGYADSVKDRSTIARDNTKNTVYLQMNSLKPEDTAVYFCAASEYDFCSTHGCYDYWGQGTQVTISL

SEQ ID NO: 214 - protein, 125 aa, Artificial Sequence
  VHH
QVQLVESGGGLVQAGGSLRLSCAASGGTFSNFNVGWFRQAPGKEREFVAASNWSAGTTHYSDSVKGRFTISRDNAANTAYLQMNSLRPDDTAVYYCNRVIRGTTYPDVYYGMDYWGKGTLVTVSS

SEQ ID NO: 215 - protein, 123 aa, Artificial Sequence
  VHH
EVQLVESGGGLVQAGGSLRLSCAASGRTFSSYGMGWFRQAPGKEREFVAAVNWSNSSAYYADSVKDRFTISSDNAKSTIYLQMNSLKPEDTAVYYCRPYSDYVTYDPDDYDYWGQGTQVTVSS

SEQ ID NO: 216 - protein, 128 aa, Artificial Sequence
  VHH
QVQLVETGGGLVQAGGSLRLSCAASGRTFSSYNMGWFRQAPGKEREFVAAISWSGGSQGYAAAVKDRFTISRDNAKNTVYLQMNSLKAEDTAVYYCAAKYHSGSYYYTSIRPEEYDYWGQGTQVTVSS

SEQ ID NO: 217 - protein, 114 aa, Artificial Sequence
  VHH
QLQLVESGGGLVQPGGSLRLSCTANGFSVGDYSMSWHRQPPGKEREVVATTARDSGSTFYAASVKGRFTISRDNAKNTVYLQMNSLKPEDTGVYYCRVNSQDYWGQGTQVTVSS

SEQ ID NO: 218 - protein, 118 aa, Artificial Sequence
  VHH
QVQLVESGGGLVQPGASLRLSCAAAGFTFSSWAMTWVRQAPGKGLEWVSAISSGSGEMADYADSVKGRFAISRDNAKNTLYLQMNNLQPEDTAMYYCAKGGYLTYANLGPGTQVTVSS

SEQ ID NO: 219 - protein, 123 aa, Artificial Sequence
  VHH
QVQLVETGGGLVQAGGSLRLSCAASGDTILFSAVGWHRQAPGKERELVAAITNSGVTYYADSVKGRFSISRDNAKNTVYLQMNSLKPEDTAVYYCNAGAPPPGEFGYDESDYWGQGTQVTVSS

SEQ ID NO: 220 - protein, 122 aa, Artificial Sequence
  VHH
EVQVVESGGGLVQPGGSLTLSCAVSGFTLDDYSIGWFRQAPGRAREAVSCTSNRDGSTYYEDSVKGRFTISRDNAKNTVYLQMNSLKPEDTAVYRCSTDCSLYGSTYSPDYWGQGTQVIVSS

SEQ ID NO: 221 - protein, 120 aa, Artificial Sequence
  VHH
QLQLVESGGGLVQPGGSLRLSCAVSGFTFSSDAMNWYRQAPGKERELVASITIDGGSTNYADSVKGRFTISRDNAKNTLYLQMNSLKPEDTAVYYCNADRGIIIYGKTYWGQGTQVTVSS

SEQ ID NO: 222 - protein, 123 aa, Artificial Sequence
  VHH
QVQLVESGGGLVQAGGSLRLSCVDSGRTFSSYGMGWFRQAPGKEREFVAAVNWRNTTAYYADSAKDRFTISSDNAKNTVYLQMASLKPEDTGVYYCRPYSDYVSYDPTEYDSWGQGTQVTVSS

SEQ ID NO: 223 - protein, 123 aa, Artificial Sequence
  VHH
EVQLVESGGGLVQPGGSLRLSCSASGDTSFISAAGWYRQAPGKERELVSAITNTGITYYPDSVKGRFTISRDNSKNTVYLQMNSLRAEDTAVYYCNAGAPPPGGLGYDESDYWGQGTQVTVSS

SEQ ID NO: 224 - protein, 123 aa, Artificial Sequence
  VHH
EVQLVESGGGLVQPGGSLRLSCSASGDTSFISAAGWYRQAPGKERELVSAITNTGITYYPDSVKGRFTISRDNAKNTVYLQMNSLRAEDTAVYYCNAGAPPPGGLGYDESDYWGQGTQVTVSS

SEQ ID NO: 225 - protein, 123 aa, Artificial Sequence
  VHH
EVQLVESGGGLVQPGGSLRLSCSASGDTSFISAAGWYRQAPGKERELVSAITNTGITYYPDSVKGRFTISRDNSKNTLYLQMNNLRAEDTAVYYCNAGAPPPGGLGYDESDYWGQGTQVTVSS

SEQ ID NO: 226 - protein, 123 aa, Artificial Sequence
  VHH
EVQLVESGGGLVQPGGSLRLSCSASGDTSFISAAGWYRQAPGKERELVSAITNTGITYYPDSVKGRFTISRDNSKNTVYLQMNNLRAEDTAVYYCNAGAPPPGGLGYDESDYWGQGTQVTVSS

SEQ ID NO: 227 - protein, 123 aa, Artificial Sequence
  VHH
EVQLVESGGGLVQPGGSLRLSCSASGDTSFISAAGWYRQAPGKERELVAAITNTGITYYPDSVKGRFTISRDNSKNTVYLQMNSLRAEDTAVYYCNAGAPPPGGLGYDESDYWGQGTLVTVSS

SEQ ID NO: 228 - protein, 124 aa, Artificial Sequence
  VHH
EVQLVESGGGLVQPGGSLRLSCAASGRPFSIYDMGWFRQAPDKERESVAVISLSRGNTYYADSVKGRFTISRDNAKNTVYLQMNSLRAEDTAVYSCGVDRRQYGLGIPPLADHWGQGTQVTVSS

SEQ ID NO: 229 - protein, 124 aa, Artificial Sequence
  VHH
EVQLVESGGGLVQPGGSLRLSCAASGRPFSIYDMGWFRQAPDKERESVAVISLSRGNTYYADSVKGRFTISRDSAKNTVYLQMNSLRAEDTAVYSCGVDRRQYGLGIPPLADHWGQGTQVTVSS

SEQ ID NO: 230 - protein, 124 aa, Artificial Sequence
  VHH
EVQLVESGGGLVQPGGSLRLSCTASGRPFSIYDMGWFRQAPDKERESVAVISLSRGNTYYADSVKGRFTISLDSAKNTVYLQMNSLRAEDTAVYSCGVDRRQYGLGIPPLADHWGQGTQVTVSS

SEQ ID NO: 231 - protein, 124 aa, Artificial Sequence
  VHH
EVQLVESGGGLVQPGGSLRLSCAASGRPFSIYDMGWFRQAPDKERESVAVINLARGNTYYADSVKGRFTISRDNAKNTVYLQMNSLRAEDTAVYSCGVDRRQYGLGIPPLADHWGQGTQVTVSS

SEQ ID NO: 232 - protein, 124 aa, Artificial Sequence
  VHH
EVQLVESGGGLVQPGGSLRLSCAASGRPFSIYDMGWFRQAPDKERESVAVINLSRGNTYYADSVKGRFTISRDNAKNTVYLQMNSLRAEDTAVYSCGVDRRQYGLGIPPLADHWGQGTQVTVSS

SEQ ID NO: 233 - protein, 124 aa, Artificial Sequence
  VHH
QVQLVESGGGSAQAGGSLRLSCTASGRPFSIYDMGWFRQAPGKERESVAVINLSRGNTYYADSVKGRFTISLDSAKNTVYLQMNSLKPEDTAVYSCGVDRRQYGLGIPPLADHWGQGTQVTVSS

SEQ ID NO: 234 - protein, 124 aa, Artificial Sequence
  VHH
QVQLVESGGGSAQAGGSLRLSCTASGRPFSIYDMGWFRQAPGKERESVAVINLSRGNTYYADSVKGRFTISLDSAKNTVYLQMNSLKPEDTAVYSCGVDRRQYGWGIPPLADHWGQGTQVTVSS

SEQ ID NO: 235 - protein, 124 aa, Artificial Sequence
  VHH
QVQLVESGGGSAQAGGSLRLSCTASGRPFSIYDMGWFRQAPGKERESVAVINLSRGNTYYADSVKGRFTISLDSAKNTVYLQMNSLKPEDTAVYSCGVDRRQYGLCIPPLADHWGQGTQVTVSS

SEQ ID NO: 236 - protein, 124 aa, Artificial Sequence
  VHH
QVQLVESGGGSAQAGGSLRLSCTASGRPFSIYDMGWFRQAPGKERESVAVINLSRGNTYYADSVKGRFTISLDSAKNTVYLQMNSLKPEDTAVYSCGVDRRQYGLDIPPLADHWGQGTQVTVSS

SEQ ID NO: 237 - protein, 124 aa, Artificial Sequence
  VHH
QVQLVESGGGSAQAGGSLRLSCTASGRPFSIYDMGWFRQAPGKERESVAVINLSRGNTYYADSVKGRFTISLDSAKNTVYLQMNSLKPEDTAVYSCGVDRRQYGLGIPHLADHWGQGTQVTVSS

SEQ ID NO: 238 - protein, 124 aa, Artificial Sequence
  VHH
QVQLVESEGGTVQAGGSLRLSCTASGRTFSGYAMGWFRQAPGKERESVAAVTLSRGNTYYADSVKGRFTISRDNAKNTFYLQMTSLKPEDTAVYHCGLDRIQYGLGIPPLADHWGQGTQVTVSS

SEQ ID NO: 239 - protein, 124 aa, Artificial Sequence
  VHH
QVQLVESGGGSAQAGGSLRLSCTASGRPFSIYDMGWFRQAPGKERESVAVINLSRGNTYYADSVKGRFTISLDSAKNTVYLQMNSLKPEDTAVYSCGVDRRQYGLGSPPLADHWGQGTQVTVSS

SEQ ID NO: 240 - protein, 124 aa, Artificial Sequence
  VHH
QVQLVESGGGSAQAGGSLRLSCTASGRPFSIYDMGWFRQAPGKERESVAVINLSRGNTYYADSVKGRFTISLDSAKNTVYLQMNSLKPEDTAVYSCGVDRRQDGLGIPPLADHWGQGTQVTVSS

SEQ ID NO: 241 - protein, 124 aa, Artificial Sequence
  VHH
QVQLVESGGGSAQAGGSLRLSCTASGRPFSIYDMGWFRQAPGKERESVAVINLSRGNTYYADSVKGRFTISLDSAKNTVYLQMNSLKPEDTAVYSCGVGRRQYGLGIPPLADHWGQGTQVTVSS

SEQ ID NO: 242 - protein, 124 aa, Artificial Sequence
  VHH
QVQLVESGGGSAQAGGSLRLSCTASGRPFSIYDMGWFRQAPGKERESVAVINLSRGNTYYADSVKGRFTISLDSAKNTVYLQMNSLKPEDTAVYSCGVDRRKYGLGIPPLADHWGQGTQVTVSS

SEQ ID NO: 243 - protein, 124 aa, Artificial Sequence
  VHH
QVQLVESGGGSAQAGGSLRLSCTASGRPFSIYDMGWFRQAPGKERESVAVINLSRGNTYYADSVKGRFTISLDSAKNTVYLQMNSLKPEDTAVYSCGVDRRQYGLGIPPPADHWGQGTQVTVSS

SEQ ID NO: 244 - protein, 124 aa, Artificial Sequence
  VHH
QVQLVESGGGSAQAGGSLRLSCTASGRPFSIYDMGWFRQAPGKERESVAVINLSRGNTYYADSVKGRFTISLDSAKNTVYLQMNSLKPEDTAVYSCGVERRQYGLGIPPLADHWGQGTQVTVSS

SEQ ID NO: 245 - protein, 124 aa, Artificial Sequence
  VHH
QVQLVESGGGSAQAGGSLRLSCTASGRPFSIYDMGWFRQAPGKERESVAVINLSRGNTYYADSVKGRFTISLDSAKNTVYLQMNSLKPEDTAVYSCGVDRRQYGFGIPPLADHWGQGTQVTVSS

SEQ ID NO: 246 - protein, 124 aa, Artificial Sequence
  VHH
QVQLVESGGGSAQAGGSLRLSCTASGRPFSIYDMGWFRQAPGKERESVAVINLSRGNTYYADSVKGRFTISLDSAKNTVYLQMNSLKPEDTAVYSCGVDRRQYGLGLPPLADHWGQGTQVTVSS

SEQ ID NO: 247 - protein, 124 aa, Artificial Sequence
  VHH
QVQLVESGGGSAQAGGSLRLSCTASGRPFSIYDMGWFRQAPGKERESVAVINLSRGNTYYADSVKGRFTISLDSAKNTVYLQMNSLKPEDTAVYSCGVDRRQYGLGIPPLADYWGQGTQVTVSS

SEQ ID NO: 248 - protein, 124 aa, Artificial Sequence
  VHH
QVQLVESGGGSAQAGGSLRLSCTASGRPFSIYDMGWFRQAPGKERESVAVINLSRGNTYYADSVKGRFTISLDSAKNTVYLQMNSLKPEDTAVYSCGVDSRQYGLGIPPLADHWGQGTQVTVSS

SEQ ID NO: 249 - protein, 124 aa, Artificial Sequence
  VHH
QVQLVESGGGSAQAGGSLRLSCTASGRPFSIYDMGWFRQAPGKERESVAVINLSRGNTYYADSVKGRFTISLDSAKNTVYLQMNSLKPEDTAVYSCGVDRRQYGLGTPPLADHWGQGTQVTVSS

SEQ ID NO: 250 - protein, 124 aa, Artificial Sequence
  VHH
QVQLVESGGGSAQAGGSLRLSCTASGRPFSIYDMGWFRQAPGKERESVAVINLSRGNTYYADSVKGRFTISLDSAKNTVYLQMNSLKPEDTAVYSCGVDRRQYGLGITPLADHWGQGTQVTVSS

SEQ ID NO: 251 - protein, 124 aa, Artificial Sequence
  VHH
QVQLVESGGGSAQAGGSLRLSCTASGRPFSIYDMGWFRQAPGKERESVAVINLSRGNTYYADSVKGRFTISLDSAKNTVYLQMNSLKPEDTAVYSCGVDRRQYRLGIPPLADHWGQGTQVTVSS

SEQ ID NO: 252 - protein, 124 aa, Artificial Sequence
  VHH
QVQLVESGGGSAQAGGSLRLSCTASGRPFSIYDMGWFRQAPGKERESVAVINLSRGNTYYADSVKGRFTISLDSAKNTVYLQMNSLKPEDTAVYSCGVDRRQYGLGNPPLADHWGQGTQVTVSS

SEQ ID NO: 253 - protein, 124 aa, Artificial Sequence
  VHH
QVQLVESGGGSAQAGGSLRLSCTASGRPFSIYDMGWFRQAPGKERESVAVINLSRGNTYYADSVKGRFTISLDSAKNTVYLQMNSLKPEDTAVYSCGVDRRQYGLGIPPLAEHWGQGTQVTVSS

SEQ ID NO: 254 - protein, 124 aa, Artificial Sequence
  VHH
QVQLVESGGGSAQAGGSLRLSCTASGRPFSIYDMGWFRQAPGKERESVAVINLSRGNTYYADSVKGRFTISLDSAKNTVYLQMNSLKPEDTAVYSCGVDRRQYGLGILPLADHWGQGTQVTVSS

SEQ ID NO: 255 - protein, 124 aa, Artificial Sequence
  VHH
QVQLVESGGGSAQAGGSLRLSCTASGRPFSIYDMGWFRQAPGKERESVAVINLSRGNTYYADSVKGRFTISLDSAKNTVYLQMNSLKPEDTAVYSCGVDRRQYGLGIHPLADHWGQGTQVTVSS

SEQ ID NO: 256 - protein, 124 aa, Artificial Sequence
  VHH
QVQLVESGGGSAQAGGSLRLSCTASGRPFSIYDMGWFRQAPGKERESVAVINLSRGNTYYADSVKGRFTISLDSAKNTVYLQMNSLKPEDTAVYSCGVDRRQYGLGVPPLADHWGQGTQVTVSS

SEQ ID NO: 257 - protein, 124 aa, Artificial Sequence
  VHH
QVQLVESGGGSAQAGGSLRLSCTASGRPFSIYDMGWFRQAPGKERESVAVINLSRGNTYYADSVKGRFTISLDSAKNTVYLQMNSLKPEDTAVYSCGVVRRQYGLGIPPLADHWGQGTQVTVSS

SEQ ID NO: 258 - protein, 124 aa, Artificial Sequence
  VHH
QVQLVESGGGSAQAGGSLRLSCTASGRPFSIYDMGWFRQAPGKERESVAVINLSRGNTYYADSVKGRFTISLDSAKNTVYLQMNSLKPEDTAVYSCGVDRRQYGLGISPLADHWGQGTQVTVSS

SEQ ID NO: 259 - protein, 124 aa, Artificial Sequence
  VHH
QVQLVESGGGSAQAGGSLRLSCTASGRPFSIYDMGWFRQAPGKERESVAVINLSRGNTYYADSVKGRFTISLDSAKNTVYLQMNSLKPEDTAVYSCEVDRRQYGLGIPPLADHWGQGTQVTVSS

SEQ ID NO: 260 - protein, 124 aa, Artificial Sequence
  VHH
QVQLVESGGGSAQAGGSLRLSCTASGRPFSIYDMGWFRQAPGKERESVAVINLSRGNTYYADSVKGRFTISLDSAKNTVYLQMNSLKPEDTAVYSCGVDKRQYGLGIPPLADHWGQGTQVTVSS

SEQ ID NO: 261 - protein, 124 aa, Artificial Sequence
  VHH
QLQLVESGGGSAQAGGSLTLSCTASGHSFSIYDMGWFRQAADKERESVAVINFGRGTTYYAESVKGRFTISLDSAKNTVYLQMNTLKPEDTAVYSCGIDRRQYGLGIPPLADHWGQGSQVTVSS

SEQ ID NO: 262 - protein, 124 aa, Artificial Sequence
  VHH
QVQLVESGGGSAQAGGSLRLSCTASGRPFSIYDMGWFRQAPGKERESVAVINLSRGNTYYADSVKGRFTISLDSAKNTVYLQMNSLKPEDTAVYSCGVDRRRYGLGIPPLADHWGQGTQVTVSS

SEQ ID NO: 263 - protein, 124 aa, Artificial Sequence
  VHH
QVQLVESGGGSAQAGGSLRLSCTASGRPFSIYDMGWFRQAPGKERESVAVINLSRGNTYYADSVKGRFTISLDSAKNTVYLQMNSLKPEDTAVYSCGVDRRQYGSGIPPLADHWGQGTQVTVSS

SEQ ID NO: 264 - protein, 124 aa, Artificial Sequence
  VHH
QVQLVESGGGSAQAGGSLRLSCTASGRPFSIYDMGWFRQAPGKERESVAVINLSRGNTYYADSVKGRFTISLDSAKNTVYLQMNSLKPEDTAVYSCGVDGRQYGLGIPPLADHWGQGTQVTVSS

SEQ ID NO: 265 - protein, 124 aa, Artificial Sequence
  VHH
QVQLVESGGGSAQAGGSLRLSCTASGRPFSIYDMGWFRQAPGKERESVAVINLSRGNTYYADSVKGRFTISLDSAKNTVYLQMNSLKPEDTAVYSCGVDRRQHGLGIPPLADHWGQGTQVTVSS

SEQ ID NO: 266 - protein, 124 aa, Artificial Sequence
  VHH
QVQLVESGGGSAQAGGSLRLSCTASGRPFSIYDMGWFRQAPGKERESVAVINLSRGNTYYADSVKGRFTISLDSAKNTVYLQMNSLKPEDTAVYSCGVDRRQYWLGIPPLADHWGQGTQVTVSS

SEQ ID NO: 267 - protein, 124 aa, Artificial Sequence
  VHH
QVQLVESGGGSAQAGGSLRLSCTASGRPFSIYDMGWFRQAPGKERESVAVINLSRGNTYYADSVKGRFTISLDSAKNTVYLQMNSLKPEDTAVYSCGVDRQQYGLGIPPLADHWGQGTQVTVSS

SEQ ID NO: 268 - protein, 124 aa, Artificial Sequence
  VHH
QVQLVESGGGSAQAGGSLRLSCTASGRPFSIYDMGWFRQAPGKERESVAVINLSRGNTYYADSVKGRFTISLDSAKNTVYLQMNSLKPEDTAVYSCGVDRWQYGLGIPPLADHWGQGTQVTVSS

SEQ ID NO: 269 - protein, 124 aa, Artificial Sequence
  VHH
QVQLVESGGGSAQAGGSLRLSCTASGRPFSIYDMGWFRQAPGKERESVAVINLSRGNTYYADSVKGRFTISLDSAKNTVYLQMNSLKPEDTAVYSCGGDRRQYGLGIPPLADHWGQGTQVTVSS

SEQ ID NO: 270 - protein, 124 aa, Artificial Sequence
  VHH
QVQLVESGGGSAQAGGSLRLSCTASGRPFSIYDMGWFRQAPGKERESVAVINLSRGNTYYADSVKGRFTISLDSAKNTVYLQMNSLKPEDTAVYSCGVNRRQYGLGIPPLADHWGQGTQVTVSS

SEQ ID NO: 271 - protein, 124 aa, Artificial Sequence
  VHH
QVQLVESGGGSAQAGGSLRLSCTASGRPFSIYDMGWFRQAPGKERESVAVINLSRGNTYYADSVKGRFTISLDSAKNTVYLQMNSLKPEDTAVYSCVVDRRQYGLGIPPLADHWGQGTQVTVSS

SEQ ID NO: 272 - protein, 124 aa, Artificial Sequence
  VHH
QVQLVESGGGSAQAGGSLRLSCTASGRPFSIYDMGWFRQAPGKERESVAVINLSRGNTYYADSVKGRFTISLDSAKNTVYLQMNSLKPEDTAVYSCGVDRRQYGLRIPPLADHWGQGTQVTVSS

SEQ ID NO: 273 - protein, 124 aa, Artificial Sequence
  VHH
QVQLVESGGGSAQAGGSLRLSCTASGGPFSIYDMGWFRQAPGKERESVAVINLSRGNTYYADSVKGRFTISLDSAKNTVYLQMNSLKPEDTAVYSCGVDRRQYGLGIPPLAAHWGQGTQVTVSS

SEQ ID NO: 274 - protein, 124 aa, Artificial Sequence
  VHH
QVQLVESGGGSAQAGGSLRLSCTASGRPFSIYDMGWFRQAPGKERESVAVINLSRGNTYYADSVKGRFTISLDSAKNTVYLQMNSLKPEDTAVYSCGVDRRQYGLGIPTLADHWGQGTQVTVSS

SEQ ID NO: 275 - protein, 124 aa, Artificial Sequence
  VHH
QVQLVESGGGSAQAGGSLRLSCTASGRPFSIYDMGWFRQAPGKERESVAVINLSRGNTYYADSVKGRFTISLDSAKNTVYLQMNSLKPEDTAVYSCGVDRLQYGLGIPPLADHWGQGTQVTVSS

SEQ ID NO: 276 - protein, 124 aa, Artificial Sequence
  VHH
QVQLVESGGGSAQAGGSLRLSCTASGRPFSIYDMGWFRQAPGKERESVAVINLSRGNTYYADSVKGRFTISLDSAKNTVYLQMNSLKPEDTAVYSCGVDRRQYGLGIRPLADHWGQGTQVTVSS

SEQ ID NO: 277 - protein, 124 aa, Artificial Sequence
  VHH
QVQLVESGGGSAQAGGSLRLSCTASGRPFSIYDMGWFRQAPGKERESVAVINLSRGNTYYADSVKGRFTISLDSAKNTVYLQMNSLKPEDTAVYSCGVDRRQYGLGFPPLADHWGQGTQVTVSS

SEQ ID NO: 278 - protein, 124 aa, Artificial Sequence
  VHH
QVQLVESGGGSAQAGGSLRLSCTASGRPFSIYDMGWFRQAPGKERESVAVINLSRGNTYYADSVKGRFTISLDSAKNTVYLQMNSLKPEDTAVYSCGADRRQYGLGIPPLADHWGQGTQVTVSS

SEQ ID NO: 279 - protein, 124 aa, Artificial Sequence
  VHH
QVQLVESGGGSAQAGGSLRLSCTASGRPFSIYDMGWFRQAPGKERESVAVINLSRGNTYYADSVKGRFTISLDSAKNTVYLQMNSLKPEDTAVYSCGVDRRQYGLSIPPLADHWGQGTQVTVSS

SEQ ID NO: 280 - protein, 124 aa, Artificial Sequence
  VHH
QVQLVESGGGSAQAGGSLRLSCTASGRPFSIYDMGWFRQAPGKERESVAVINLSRGNTYYADSVKGRFTISLDSAKNTVYLQMNSLKPEDTAVYSCGVDIRQYGLGIPPLADHWGQGTQVTVSS

SEQ ID NO: 281 - protein, 124 aa, Artificial Sequence
  VHH
QVQLVESGGGLVQAGGSLRLSCTASGLTFSTYAMGWFRQAPGNERESVAAINLSRGNTYYADSVKGRFTISRDNAKNTVYLQMNSLKPEDTAVYHCGVDKIQYGLGLPVLADHWGQGTQVTVSS

SEQ ID NO: 282 - protein, 124 aa, Artificial Sequence
  VHH
QVQLVESGGGSAQAGGSLRLSCTASGRPFSIYDMGWFRQAPGKERESVAVINLSRGNTYYADSVKGRFTISLDSAKNTVYLQMNSLKPEDTAVYSCGVDRRQYGLGIPPRADHWGQGTQVTVSS

SEQ ID NO: 283 - protein, 124 aa, Artificial Sequence
  VHH
QVQLVESGGGSAQAGGSLRLSCTASGRPFSIYDMGWFRQAPGKERESVAVINLSRGNTYYADSVKGRFTISLDSAKNTVYLQMNSLKPEDTAVYSCGVDRRQYGLGIPPFADHWGQGTQVTVSS

SEQ ID NO: 284 - protein, 124 aa, Artificial Sequence
  VHH
QVQLVESGGGSAQAGGSLRLSCTASGRPFSIYDMGWFRQAPGKERESVAVINLSRGNTYYADSVKGRFTISLDSAKNTVYLQMNSLKPEDTAVYSCGVDRRQYGLGIPPLADRWGQGTQVTVSS

SEQ ID NO: 285 - protein, 124 aa, Artificial Sequence
  VHH
QVQLVESGGGSAQAGGSLRLSCTASGRPFSIYDMGWFRQAPGKERESVAVINLSRGNTYYADSVKGRFTISLDSAKNTVYLQMNSLKPEDTAVYSCGVDRRQYGLGIPPLAGHWGQGTQVTVSS

SEQ ID NO: 286 - protein, 124 aa, Artificial Sequence
  VHH
QVQLVESGGGSAQAGGSLRLSCTASGRPFSIYDMGWFRQAPGKERESVAVINLSRGNTYYADSVKGRFTISLDSAKNTVYLQMNSLKPEDTAVYSCGVDRRQYGVGIPPLADHWGQGTQVTVSS

SEQ ID NO: 287 - protein, 124 aa, Artificial Sequence
  VHH
EVQLVESGGGSAQAGGSLRLSCTASGRPFSIYDMGWFRQAPGKERESVAVINLSRGNTYYADSVKGRFTISLDSAKNTVYLQMNSLKPEDTAVYSCGVDRRQYGLGIPPHADHWGQGTQVTVSS

SEQ ID NO: 288 - protein, 124 aa, Artificial Sequence
  VHH
QVQLVESGGGSAQAGGSLRLSCTASGRPFSIYDMGWFRQAPGKERESVAVINLSRGNTYYADSVKGRFTISLDSAKNTVYLQMNSLKPEDTAVYSCGVARRQYGLGIPPLADHWGQGTQVTVSS

SEQ ID NO: 289 - protein, 124 aa, Artificial Sequence
  VHH
QVQLVESGGGSAQAGGSLRLSCTASGRPFSIYDMGWFRQAPGKERESVAVINLSRGNTYYADSVKGRFTISLDSAKNTVYLQMNSLKPEDTAVYSCGVYRRQYGLGIPPLADHWGQGTQVTVSS

SEQ ID NO: 290 - protein, 124 aa, Artificial Sequence
  VHH
QVQLVESGGGSAQAGGSLRLSCTASGHSFSIYDMGWFRQAPGKERESVAVINLSRGNTYYADSVKGRFTISLDSAKNTVYLQMNSLKPEDTAVYSCGVDRCQYGLGIPPLADHWGQGTQVTVSS

SEQ ID NO: 291 - protein, 124 aa, Artificial Sequence
  VHH
QVQLVESGGGSAQAGGSLRLSCTASGRPFSIYDMGWFRQAPGKERESVAVINLSRGNTYYADSVKGRFTISLDSAKNTVYLQMNSLKPEDTAVYSCGVDRRQCGLGIPPLADHWGQGTQVTVSS

SEQ ID NO: 292 - protein, 124 aa, Artificial Sequence
  VHH
EVQVVESGGGSAQAGGSLRLSCTASGRPFSIYDMGWFRQAPGKERESVAVINLSRGNTYYADSVKGRFTISLDSAKNTVYLQMNSLKPEDTAVYSCGVDRRQYGLGIPPLVDHWGQGTQVTVSS

SEQ ID NO: 293 - protein, 124 aa, Artificial Sequence
  VHH
QVQLVETGGGSAQAGGSLRLSCTASGRPFSIYDMGWFRQAPGKERESVAVINLSRGNTYYADSVKGRFTISLDSAKNTVYLQMNSLKPEDTAVYSCGVDRRPYGLGIPPLADHWGQGTQVTVSS

SEQ ID NO: 294 - protein, 124 aa, Artificial Sequence
  VHH
EVQLVESGGGSAQAGGSLRLSCTASGRPFSIYDMGWFRQAPGKERESVAVINLSRGNTYYADSVKGRFTISLDSAKNTVYLQMNSLKPEDTAVYSCGVDRRQYGLGIPPLADNWGQGTQVTVSS

SEQ ID NO: 295 - protein, 124 aa, Artificial Sequence
  VHH
QVQLVESEGGTVQAGGSLRLSCTASGRTFSGYAMGWFRQAPGKERESVAAVTLSRGNTYYADSVKGRFTISRDNAKNTFYLQMTSLKPEDTAVYHCGLDRIQYGLGIPPLADYWGQGTQVTVSS

SEQ ID NO: 296 - protein, 124 aa, Artificial Sequence
  VHH
QVQLVESGGGSAQAGGSLRLSCTASGGPFSIYDMGWFRQAPGKERESVAVINLSRGNTYYADSVKGRFTISLDSAKNTVYLQMNSLKPEDTAVYSCGLDRRQYGLGIPPLADHWGQGTQVTVSS

SEQ ID NO: 297 - protein, 124 aa, Artificial Sequence
  VHH
QVQLVESGGGSAQAGGSLRLSCTASGHSFSIYDMGWFRQAPGKERESVAVINLSRGNTYYADSVKGRFTISLDSAKNTVYLQMNSLKPEDTAVYSCGVDRRQYGLGIPPLADQWGQGTQVTVSS

SEQ ID NO: 298 - protein, 124 aa, Artificial Sequence
  VHH
QVQLVESGGGSAQAGGSLRLSCTASGRPFSIYDMGWFRQAPGKERESVAVINLSRGNTYYADSVKGRFTISLDSAKNTVYLQMNSLKPEDTAVYSCGVDRRQYGLGIPPIADHWGQGTQVTVSS

SEQ ID NO: 299 - protein, 124 aa, Artificial Sequence
  VHH
QVQLVESGGGSAQAGGSLRLSCTASGRPFSIYDMGWFRQAPGKERESVAVINLSRGNTYYADSVKGRFTISLDSAKNTVYLQMNSLKPEDTAVYSCGVDRRQYGLVIPPLADHWGQGTQVTVSS

SEQ ID NO: 300 - protein, 124 aa, Artificial Sequence
  VHH
QVQLVESGGGSAQAGGSLRLSCTASGGPFSIYDMGWFRQAPGKERESVAVINLSRGNTYYADSVKGRFTISLDSAKNTVYLQMNSLKPEDTAVYSCGVDRRQYVLGIPPLADHWGQGTQVTVSS

SEQ ID NO: 301 - protein, 124 aa, Artificial Sequence
  VHH
QVQLVESGGGSAQAGGSLRLSCTASGGPFSIYDMGWFRQAPGKERESVAVINLSRGNTYYADSVKGRFTISLDSAKNTVYLQMNSLKPEDTAVYSCGVDRRQYGLGIPPLSDHWGQGTQVTVSS

SEQ ID NO: 302 - protein, 124 aa, Artificial Sequence
  VHH
QVQLVESEGGTVQAGGSLRLSCTASGRTFSGYAMGWFRQAPGKERESVAAVTLSRGNTYYADSVKGRFTISRDNAKNTFYLQMTSLKPEDTAVYHCGIDRIQYGLGIPPLADHWGQGTQVTVSS

SEQ ID NO: 303 - protein, 124 aa, Artificial Sequence
  VHH
EVQLVESGGGSAQAGGSLRLSCTASGRPFSIYDMGWFRQAPGKERESVAVINLSRGNTYYADSVKGRFTISLDSAKNTVYLQMNSLKPEDTAVYSCGVDRREYGLGIPPLADHWGQGTQVTVSS

SEQ ID NO: 304 - protein, 124 aa, Artificial Sequence
  VHH
QVQLVESGGGSAQAGGSLRLSCTASGRPFSIYDMGWFRQAPGKERESVAVINLSRGNTYYADSVKGRFTISLDSAKNTVYLQMNSLKPEDTAVYSCGVDRRQYGLGIPSLADHWGQGTQVTVSS

SEQ ID NO: 305 - protein, 124 aa, Artificial Sequence
  VHH
EVQVVESGGGSAQAGGSLRLSCTASGRPFSIYDMGWFRQAPGKERESVAVINLSRGNTYYADSVKGRFTISLDSAKNTVYLQMNSLKPEDTAVYSCGVDRRQYGLGIPPLAHHWGQGTQVTVSS

SEQ ID NO: 306 - protein, 124 aa, Artificial Sequence
  VHH
QVQLVESGGGSAQAGGSLRLSCTASGRPFSIYDMGWFRQAPGKERESVAVINLSRGNTYYADSVKGRFTISLDSAKNTVYLQMNSLKPEDTAVYSCGVDRRQNGLGIPPLADHWGQGTQVTVSS

SEQ ID NO: 307 - protein, 124 aa, Artificial Sequence
  VHH
QVQLVESGGGSAQAGGSLRLSCTASGRPFSIYDMGWFRQAPGKERESVAVINLSRGNTYYADSVKGRFTISLDSAKNTVYLQMNSLKPEDTAVYSCGVDRRQYGLGIPPLAVHWGQGTQVTVSS

SEQ ID NO: 308 - protein, 124 aa, Artificial Sequence
  VHH
QVQLVESGGGSAQAGGSLRLSCTASGRPFSIYDMGWFRQAPGKERESVAVINLSRGNTYYADSVKGRFTISLDSAKNTVYLQMNSLKPEDTAVYSCGVDRRQYGWCIPPLADHWGQGTQVTVSS

SEQ ID NO: 309 - protein, 124 aa, Artificial Sequence
  VHH
QVQLVESGGGSAQAGGSLRLSCTASGRPFSIYDMGWFRQAPGKERESVAVINLSRGNTYYADSVKGRFTISLDSAKNTVYLQMNSLKPEDTAVYSCGVDRRQYELGIPPLADHWGQGTQVTVSS

SEQ ID NO: 310 - protein, 124 aa, Artificial Sequence
  VHH
QVQLVESGGGLVQPGGSLRLSCSASGHSFSIYDMGWFRQAADKERESVAVINFGRGTTYYAESVKGRFTISRDNAKNTVYLQMNSLRAEDTAVYSCGIDRRQYGLGIPPLADHWGQGSQVTVSS

SEQ ID NO: 311 - protein, 124 aa, Artificial Sequence
  VHH
QLQLVESGGGLVQPGGSLRLSCSASGHSFSIYDMGWFRQAADKERESVAVINFGRGTTYYAESVKGRFTISRDNAKNTVYLQMNSLRAEDTAVYSCGIDRRQYGLGIPPLADHWGQGSQVTVSS

SEQ ID NO: 312 - protein, 124 aa, Artificial Sequence
  VHH
QVQLVESGGGLVQPGGSLTLSCSASGHSFSIYDMGWFRQAADKERESVAVINFGRGTTYYAESVKGRFTISRDNAKNTVYLQMNSLRAEDTAVYSCGIDRRQYGLGIPPLADHWGQGSQVTVSS

SEQ ID NO: 313 - protein, 124 aa, Artificial Sequence
  VHH
QVQLVESGGGLVQPGGSLRLSCTASGHSFSIYDMGWFRQAADKERESVAVINFGRGTTYYAESVKGRFTISRDNAKNTVYLQMNSLRAEDTAVYSCGIDRRQYGLGIPPLADHWGQGSQVTVSS

SEQ ID NO: 314 - protein, 124 aa, Artificial Sequence
  VHH
QVQLVESGGGLVQPGGSLRLSCSASGHSFSIYDMGWFRQAPDKERESVAVINFGRGTTYYAESVKGRFTISRDNAKNTVYLQMNSLRAEDTAVYSCGIDRRQYGLGIPPLADHWGQGSQVTVSS

SEQ ID NO: 315 - protein, 124 aa, Artificial Sequence
  VHH
QVQLVESGGGLVQPGGSLRLSCSASGHSFSIYDMGWFRQAAGKERESVAVINFGRGTTYYAESVKGRFTISRDNAKNTVYLQMNSLRAEDTAVYSCGIDRRQYGLGIPPLADHWGQGSQVTVSS

SEQ ID NO: 316 - protein, 124 aa, Artificial Sequence
  VHH
QVQLVESGGGLVQPGGSLRLSCSASGHSFSIYDMGWFRQAADKERESVAVINFGRGTTYYAESVKGRFTISLDNAKNTVYLQMNSLRAEDTAVYSCGIDRRQYGLGIPPLADHWGQGSQVTVSS

SEQ ID NO: 317 - protein, 124 aa, Artificial Sequence
  VHH
QVQLVESGGGLVQPGGSLRLSCSASGHSFSIYDMGWFRQAPGKERESVAVINFGRGTTYYAESVKGRFTISRDNAKNTVYLQMNSLRAEDTAVYSCGIDRRQYGLGIPPLADHWGQGSQVTVSS

SEQ ID NO: 318 - protein, 124 aa, Artificial Sequence
  VHH
QVQLVESGGGLVQPGGSLRLSCSASGFTFSIYDMGWFRQAADKERESVAVINFGRGTTYYAESVKGRFTISRDNAKNTVYLQMNSLRAEDTAVYSCGIDRRQYGLGIPPLADHWGQGSQVTVSS

SEQ ID NO: 319 - protein, 124 aa, Artificial Sequence
  VHH
ELQLVESGGGLVQPGGSLRLSCAASGHSFSIYDMGWFRQAADKERESVAVINFGRGTTYYAESVKGRFTISRDNAKNTVYLQMNSLRAEDTAVYSCGIDRRQYGLGIPPLADHWGQGSQVTVSS

SEQ ID NO: 320 - protein, 8 aa, Artificial Sequence
  CDR1
GFTFSIYD

SEQ ID NO: 321 - protein, 229 aa, Artificial Sequence
  CH
ESKYGPPCPPCPAPEFLGGPSVFLFPPKPKDTLMISRTPEVTCVVVDVSQEDPEVQFNWYVDGVEVHNAKTKPREEQFNSTYRVVSVLTVLHQDWLNGKEYKCKVSNKGLPSSIEKTISKAKGQPREPQVYTLPPSQEEMTKNQVSLTCLVKGFYPSDIAVEWESNGQPENNYKTTPPVLDSDGSFFLYSRLTVDKSRWQEGNVFSCSVMHEALHNHYTQKSLSLSLGK

SEQ ID NO: 322 - DNA, 369 bp, Artificial Sequence
  VHH
caggtgcagctcgtggagtctgggggaggcttggtgcaggctgggggctctctgagactctcctgtgcagcctctggagacaccagctttatttctgccgcgggctggtaccgccaggctccagggaaggagcgcgaattggtcgcagcgattactaatactggtatcacatactatccagactccgtgaagggccgattcaccatctccagagacaatgccaaaaacacggtgtatctgcaaatgaacaacctgaaacctgaggacacggccgtctattactgtaacgcaggagcccctcctcctggcgggttggggtatgatgaatccgactactggggccaggggacccaggtcaccgtctcctca

SEQ ID NO: 323 - DNA, 372 bp, Artificial Sequence
  VHH
caggtgcagctggtggagactgggggaggattggtgcgggctgggggctctctgagactctcctgtacagcctctggacgccccttcagtatttatgacatgggctggttccgccaggctccagacaaagagcgtgagtcggtagcagtaattaatttgagtcgtggtgacacatactatgcagactccgtgaagggccgattcaccatctccctcgactccgccaagaacacggtgtatctgcagatgaacagcctgaaacctgaggacacggccgtttatagctgtggagtagatagacgtcagtacggattgggcatccccccccttgctgaccactggggccaggggacccaggtcaccgtctcctca

SEQ ID NO: 324 - DNA, 24 bp, Artificial Sequence
  primer
gtcctggctgctcttctacaaggc

SEQ ID NO: 325 - DNA, 23 bp, Artificial Sequence
  primer
ggtacgtgctgttgaactgttcc

SEQ ID NO: 326 - DNA, 29 bp, Artificial Sequence
  primer
gatgtgcagctgcaggagtctggrggagg

SEQ ID NO: 327 - DNA, 35 bp, Artificial Sequence
  primer
ggactagtgcggccgctggagacggtgacctgggt